European Patent Specification EP 4 059 951 B1, published October 29, 2025. Title: Novel membrane protein TerC variant and a method for producing L-lysine using the same. Applicant: CJ CheilJedang Corporation. The sequence listing filed with the application follows.

SEQUENCE LISTING (10 sequences)

SEQ ID NO: 1 - protein, 369 aa, Artificial Sequence
  (E294K)_membrane protein TerC
MEVNLATWLITIAVIAGFFIFDFYSHVRTPHEPTIKESAWWSLFYVALACVFGVFLWFAWGEPGNPHQHGIEFFTGYVTEKALSVDNLFIFALIMGSFKIPRKYQQKVLLIGIALALVFRLAFILAGAAVIEAWSDVFYIFSIWLIYTAVKLLWDEVRDTPETDPNDMFIIKALRKVIPVTEGYHGDKLTHRFGGKLHLTPLFVALVSIGMVDLMFALDSIPAIYGITTEPYIVFTTNAFALLGLRQMYFLLDGLLDRLVYLPYGLGLILLFIGAKLGLHALHENNLPFINGGKNVSVPEVSTVFSLVFIIGVLTITVIASIIKNKRDENQGGIPPKWNAAKYEGDNWETGEEPETGSATVTDISSEKK

SEQ ID NO: 2 - DNA, 1110 bp, Artificial Sequence
  (E294K)_NCgl1892
atggaagtaaacttagccacatggctaatcactatcgcagtgattgctggcttcttcattttcgatttctattcccacgtccgcaccccacacgagcccactatcaaagaatccgcatggtggagcctcttctacgtagccctcgcctgtgttttcggcgtgttcctctggtttgcttggggcgagccaggtaacccacaccagcacggcattgagttcttcaccggttacgtgacagagaaggcgttgagtgttgataacctcttcatcttcgcgctgatcatgggttctttcaagattcctcgcaagtaccagcagaaggttctgctcatcggtatcgcgctggcactggtcttccgcctggcattcatcctcgcaggtgctgcagttatcgaagcctggtccgatgtcttctacatcttctccatctggctgatctacaccgctgtgaagctcctgtgggacgaagttcgagacacccctgagaccgacccgaacgacatgttcatcattaaggcgctgcgcaaggtcattccggttactgagggctaccacggcgacaagctcactcaccgcttcggaggcaagctgcacctgaccccactgttcgttgcacttgtatccatcggcatggttgacctgatgttcgcactggactctatcccagcgatttacggcatcaccacggagccttacatcgtgttcaccactaacgcattcgccctgctgggtctgcgccaaatgtacttcctgcttgacggcctgcttgaccgcctggtctacctgccttatggcttgggtcttatcctgctgttcattggtgcaaagcttggtctgcatgcactgcacgaaaacaacctgccattcatcaacggtggtaaaaacgtctccgtacctgaggtttccaccgtgttctccttggtcttcatcattggtgtcctgacaatcaccgtcatcgcatccatcatcaagaacaaacgcgacgaaaaccagggcggtattccaccaaagtggaacgctgcaaagtatgagggcgacaactgggagaccggtgaggagcctgaaaccggatccgccaccgttaccgatatctcctcagagaagaagtaa

SEQ ID NO: 3 - protein, 369 aa, Artificial Sequence
  (WT)_membrane protein TerC
MEVNLATWLITIAVIAGFFIFDFYSHVRTPHEPTIKESAWWSLFYVALACVFGVFLWFAWGEPGNPHQHGIEFFTGYVTEKALSVDNLFIFALIMGSFKIPRKYQQKVLLIGIALALVFRLAFILAGAAVIEAWSDVFYIFSIWLIYTAVKLLWDEVRDTPETDPNDMFIIKALRKVIPVTEGYHGDKLTHRFGGKLHLTPLFVALVSIGMVDLMFALDSIPAIYGITTEPYIVFTTNAFALLGLRQMYFLLDGLLDRLVYLPYGLGLILLFIGAKLGLHALHENNLPFINGGENVSVPEVSTVFSLVFIIGVLTITVIASIIKNKRDENQGGIPPKWNAAKYEGDNWETGEEPETGSATVTDISSEKK

SEQ ID NO: 4 - DNA, 1110 bp, Artificial Sequence
  (WT)_NCgl1892
atggaagtaaacttagccacatggctaatcactatcgcagtgattgctggcttcttcattttcgatttctattcccacgtccgcaccccacacgagcccactatcaaagaatccgcatggtggagcctcttctacgtagccctcgcctgtgttttcggcgtgttcctctggtttgcttggggcgagccaggtaacccacaccagcacggcattgagttcttcaccggttacgtgacagagaaggcgttgagtgttgataacctcttcatcttcgcgctgatcatgggttctttcaagattcctcgcaagtaccagcagaaggttctgctcatcggtatcgcgctggcactggtcttccgcctggcattcatcctcgcaggtgctgcagttatcgaagcctggtccgatgtcttctacatcttctccatctggctgatctacaccgctgtgaagctcctgtgggacgaagttcgagacacccctgagaccgacccgaacgacatgttcatcattaaggcgctgcgcaaggtcattccggttactgagggctaccacggcgacaagctcactcaccgcttcggaggcaagctgcacctgaccccactgttcgttgcacttgtatccatcggcatggttgacctgatgttcgcactggactctatcccagcgatttacggcatcaccacggagccttacatcgtgttcaccactaacgcattcgccctgctgggtctgcgccaaatgtacttcctgcttgacggcctgcttgaccgcctggtctacctgccttatggcttgggtcttatcctgctgttcattggtgcaaagcttggtctgcatgcactgcacgaaaacaacctgccattcatcaacggtggtgaaaacgtctccgtacctgaggtttccaccgtgttctccttggtcttcatcattggtgtcctgacaatcaccgtcatcgcatccatcatcaagaacaaacgcgacgaaaaccagggcggtattccaccaaagtggaacgctgcaaagtatgagggcgacaactgggagaccggtgaggagcctgaaaccggatccgccaccgttaccgatatctcctcagagaagaagtaa

SEQ ID NO: 5 - DNA, 40 bp, Artificial Sequence
  NCgl1892_1F
tgaattcgagctcggtacccttcatcctcgcaggtgctgc

SEQ ID NO: 6 - DNA, 33 bp, Artificial Sequence
  NCgl1892_2R
ggtacggagacgtttttaccaccgttgatgaat

SEQ ID NO: 7 - DNA, 33 bp, Artificial Sequence
  NCgl1892_3F
attcatcaacggtggtaaaaacgtctccgtacc

SEQ ID NO: 8 - DNA, 40 bp, Artificial Sequence
  NCgl1892_4R
gtcgactctagaggatccccatgaacaatgatccattcca

SEQ ID NO: 9 - DNA, 20 bp, Artificial Sequence
  NCgl1892_5F
ttcatcctcgcaggtgctgc

SEQ ID NO: 10 - DNA, 20 bp, Artificial Sequence
  NCgl1892_6R
atgaacaatgatccattcca